European Patent Specification EP 3 732 190 B1, published August 6, 2025. Title: RECOMBINANT POLYPEPTIDES AND METHODS OF USE THEREOF. Applicant: Imunami Laboratories Pte. Ltd. The sequence listing filed with the application follows.

SEQUENCE LISTING (52 sequences)

SEQ ID NO: 1 - protein, 173 aa, Anser cygnoides
MDITIQHPWFKRALGPLIPSRLFDQFFGEGLLEYDLLPLFSSTISPYYRQSLFRSVLESGISEVRSDRDKFTIMLDVKHFSPEDLSVKIIDDFVEIHGKHSERQDDHGYISREFHRRYRLPANVDQSAITCSLSGDGMLTFSGPKVPSNMDPTHSERPIPVSREEKPTSAPSS

SEQ ID NO: 2 - protein, 173 aa, Rhea americana
MDITIQHPWFKRALGPLIPSRLFDQFFGEGLLEYDLLPLFSSTISPYYRQSLFRSVLESGISEVRSDREKFTIMLDVKHFSPEDLSVKIIDDFVEIHGKHSERQDDHGYISREFHRRYRLPSNVDQSAITCSLSSDGMLTFSGPKVQANMDPSHSERPIPVSREEKPTSAPSS

SEQ ID NO: 3 - protein, 149 aa, Anas platyrhynchos
RALGPLIPSRLFDQFFGEGLLEYDLLPLFSSTISPYYRQSLFRSVLESGISEVRSDRDKFTIMLDVKHFSPEDLSVKIIDDFVEIHGKHSERQDDHGYISREFHRRYRLPANVDQSAITCSLSGDGMLTFSGPKVPSNMDPTHSERPIP

SEQ ID NO: 4 - protein, 174 aa, Anas platyrhynchos
MDITIHNPLIRRPLFSWLAPSRIFDQIFGEHLQESELLPASPSLSPFLMRSPIFRMPSWLETGLSEMRLEKDKFSVNLDVKHFSPEELKVKVLGDMVEIHGKHEERQDEHGFIAREFNRKYRIPADVDPLTITSSLSLDGVLTVSAPRKQSDVPERSIPITREEKPAIAGAQRK

SEQ ID NO: 5 - protein, 173 aa, Homo sapiens
MDVTIQHPWFKRTLGPFYPSRLFDQFFGEGLFEYDLLPFLSSTISPYYRQSLFRTVLDSGISEVRSDRDKFVIFLDVKHFSPEDLTVKVQDDFVEIHGKHNERQDDHGYISREFHRRYRLPSNVDQSALSCSLSADGMLTFCGPKIQTGLDATHAERAIPVSREEKPTSAPSS

SEQ ID NO: 6 - protein, 186 aa, Drosophila melanogaster
MANIPLLLSLADDLGRMSMVPFYEPYYCQRQRNPYLALVGPMEQQLRQLEKQVGASSGSSGAVSKIGKDGFQVCMDVSHFKPSELVVKVQDNSVLVEGNHEEREDDHGFITRHFVRRYALPPGYEADKVASTLSSDGVLTIKVPKPPAIEDKGNERIVQIQQVGPAHLNVKENPKEAVEQDNGNDK

SEQ ID NO: 7 - protein, 174 aa, Drosophila melanogaster
MRSLPMFWRMAEEMARMPRLSSPFHAFFHEPPVWSVALPRNWQHIARWQEQELAPPATVNKDGYKLTLDVKDYSELKVKVLDESVVLVEAKSEQQEAEQGGYSSRHFLGRYVLPDGYEADKVSSSLSDDGVLTISVPNPPGVQETLKEREVTIEQTGEPAKKSAEEPKDKTASQ

SEQ ID NO: 8 - protein, 174 aa, Anser cygnoides; identical to SEQ ID NO: 4

SEQ ID NO: 9 - protein, 173 aa, Artificial Sequence
  artificial polypeptide
MDITIQHPWFKRALGPLIPERLFDQFFGSGLLSYDLLPLFEETIEPYYRQELFREVLSEGIESVREDRDKFTIMLDVKHFEPSDLEVKIIDDFVSIHGKHESRQDDHGYIERSFHRRYRLPANVDQEAITCELEGDGMLTFEGPKVPENMDPTHESRPIPVERSSKPTEAPEE

SEQ ID NO: 10 - protein, 173 aa, Artificial Sequence
  artificial polypeptide
MDITIQHPWFKRALGPLIPERLFDQFFGSGLLSYDLLPLFEETIEPYYRQELFREVLSEGIESVREDRSKFTIMLDVKHFEPSDLEVKIIDDFVSIHGKHESRQDDHGYIERSFHRRYRLPENVDQEAITCELEEDGMLTFEGPKVQANMDPEHESRPIPVERSSKPTEAPEE

SEQ ID NO: 11 - protein, 149 aa, Artificial Sequence
  artificial polypeptide
RALGPLIPERLFDQFFGSGLLSYDLLPLFEETIEPYYRQELFREVLSEGIESVREDRDKFTIMLDVKHFEPSDLEVKIIDDFVSIHGKHESRQDDHGYIERSFHRRYRLPANVDQEAITCELEGDGMLTFEGPKVPENMDPTHESRPIP

SEQ ID NO: 12 - protein, 174 aa, Artificial Sequence
  artificial polypeptide
MSITIHNPLIRRPLFDWLAPDRIFSQIFGEHLQEDELLPADPDLDPFLMRDPIFRMPDWLETGLDEMRLEKSKFDVNLSVKHFDPEELKVKVLGSMVEIHGKHEERQSEHGFIAREFNRKYRIPASVSPLTITDDLDLSGVLTVDAPRKQDSVPERDIPITREEKPAIAGAQRK

SEQ ID NO: 13 - protein, 173 aa, Artificial Sequence
  artificial polypeptide
MDVTIQHPWFKRTLGPFYPERLFDQFFGSGLFSYDLLPFLEETIEPYYRQELFRTVLDEGIESVREDRDKFVIFLDVKHFEPSDLTVKVQDDFVSIHGKHNSRQDDHGYIERSFHRRYRLPENVDQEALECELEADGMLTFCGPKIQTGLDATHASRAIPVERSSKPTEAPEE

SEQ ID NO: 14 - protein, 186 aa, Artificial Sequence
  artificial polypeptide
MANIPLLLSLAVVLGRMSMDPFYEPYYCQRQRNPYLALDGPMEQQLRQLEKQDGASSGSSGADSKIGKVGFQDCMVDSHFKPSELDDKDQVNSDLDEGNHEEREVVHGFITRHFDRRYALPPGYEAVKDASTLSSVGDLTIKDPKPPAIEVKGNERIDQIQQDGPAHLNDKENPKEADEQVNGNVK

SEQ ID NO: 15 - protein, 174 aa, Artificial Sequence
  artificial polypeptide
MRLSPMFWRMAEEMARMPRSLLPFHAFFHEPPDWLDASPRNWQHIARWQEQESAPPATDNKVGYKSTSVDKVYLESKDKDSVELDDSDEAKLEQQEAEQGGYLLRHFSGRYDSPVGYEAVKDLLLSLVVGDSTILDPNPPGDQETSKEREDTIEQTGEPAKKLAEEPKVKTALQ

SEQ ID NO: 16 - protein, 174 aa, Artificial Sequence; identical to SEQ ID NO: 12
  artificial polypeptide

SEQ ID NO: 17 - DNA, 519 bp, Anser cygnoides
atggatattaccattcagcatccgtggtttaaacgcgcgctgggcccgctgattccgagccgcctgtttgatcagttttttggcgaaggcctgctggaatatgatctgctgccgctgtttagcagcaccattagcccgtattatcgccagagcctgtttcgcagcgtgctggaaagcggcattagcgaagtgcgcagcgatcgcgataaatttaccattatgctggatgtgaaacattttagcccggaagatctgagcgtgaaaattattgatgattttgtggaaattcatggcaaacatagcgaacgccaggatgatcatggctatattagccgcgaatttcatcgccgctatcgcctgccggcgaacgtggatcagagcgcgattacctgcagcctgagcggcgatggcatgctgacctttagcggcccgaaagtgccgagcaacatggatccgacccatagcgaacgcccgattccggtgagccgcgaagaaaaaccgaccagcgcgccgagcagc

SEQ ID NO: 18 - DNA, 519 bp, Rhea americana
atggatattaccattcagcatccgtggtttaaacgcgcgctgggcccgctgattccgagccgcctgtttgatcagttttttggcgaaggcctgctggaatatgatctgctgccgctgtttagcagcaccattagcccgtattatcgccagagcctgtttcgcagcgtgctggaaagcggcattagcgaagtgcgcagcgatcgcgaaaaatttaccattatgctggatgtgaaacattttagcccggaagatctgagcgtgaaaattattgatgattttgtggaaattcatggcaaacatagcgaacgccaggatgatcatggctatattagccgcgaatttcatcgccgctatcgcctgccgagcaacgtggatcagagcgcgattacctgcagcctgagcagcgatggcatgctgacctttagcggcccgaaagtgcaggcgaacatggatccgagccatagcgaacgcccgattccggtgagccgcgaagaaaaaccgaccagcgcgccgagcagc

SEQ ID NO: 19 - DNA, 447 bp, Anas platyrhynchos
cgcgcgctgggcccgctgattccgagccgcctgtttgatcagttttttggcgaaggcctgctggaatatgatctgctgccgctgtttagcagcaccattagcccgtattatcgccagagcctgtttcgcagcgtgctggaaagcggcattagcgaagtgcgcagcgatcgcgataaatttaccattatgctggatgtgaaacattttagcccggaagatctgagcgtgaaaattattgatgattttgtggaaattcatggcaaacatagcgaacgccaggatgatcatggctatattagccgcgaatttcatcgccgctatcgcctgccggcgaacgtggatcagagcgcgattacctgcagcctgagcggcgatggcatgctgacctttagcggcccgaaagtgccgagcaacatggatccgacccatagcgaacgcccgattccg

SEQ ID NO: 20 - DNA, 522 bp, Anas platyrhynchos
atggatattaccattcataacccgctgattcgccgcccgctgtttagctggctggcgccgagccgcatttttgatcagatttttggcgaacatctgcaggaaagcgaactgctgccggcgagcccgagcctgagcccgtttctgatgcgcagcccgatttttcgcatgccgagctggctggaaaccggcctgagcgaaatgcgcctggaaaaagataaatttagcgtgaacctggatgtgaaacattttagcccggaagaactgaaagtgaaagtgctgggcgatatggtggaaattcatggcaaacatgaagaacgccaggatgaacatggctttattgcgcgcgaatttaaccgcaaatatcgcattccggcggatgtggatccgctgaccattaccagcagcctgagcctggatggcgtgctgaccgtgagcgcgccgcgcaaacagagcgatgtgccggaacgcagcattccgattacccgcgaagaaaaaccggcgattgcgggcgcgcagcgcaaa

SEQ ID NO: 21 - DNA, 519 bp, Homo sapiens
atggatgtgaccattcagcatccgtggtttaaacgcaccctgggcccgttttatccgagccgcctgtttgatcagttttttggcgaaggcctgtttgaatatgatctgctgccgtttctgagcagcaccattagcccgtattatcgccagagcctgtttcgcaccgtgctggatagcggcattagcgaagtgcgcagcgatcgcgataaatttgtgatttttctggatgtgaaacattttagcccggaagatctgaccgtgaaagtgcaggatgattttgtggaaattcatggcaaacataacgaacgccaggatgatcatggctatattagccgcgaatttcatcgccgctatcgcctgccgagcaacgtggatcagagcgcgctgagctgcagcctgagcgcggatggcatgctgaccttttgcggcccgaaaattcagaccggcctggatgcgacccatgcggaacgcgcgattccggtgagccgcgaagaaaaaccgaccagcgcgccgagcagc

SEQ ID NO: 22 - DNA, 558 bp, Drosophila melanogaster
atggcgaacattccgctgctgctgagcctggcggatgatctgggccgcatgagcatggtgccgttttatgaaccgtattattgccagcgccagcgcaacccgtatctggcgctggtgggcccgatggaacagcagctgcgccagctggaaaaacaggtgggcgcgagcagcggcagcagcggcgcggtgagcaaaattggcaaagatggctttcaggtgtgcatggatgtgagccattttaaaccgagcgaactggtggtgaaagtgcaggataacagcgtgctggtggaaggcaaccatgaagaacgcgaagatgatcatggctttattacccgccattttgtgcgccgctatgcgctgccgccgggctatgaagcggataaagtggcgagcaccctgagcagcgatggcgtgctgaccattaaagtgccgaaaccgccggcgattgaagataaaggcaacgaacgcattgtgcagattcagcaggtgggcccggcgcatctgaacgtgaaagaaaacccgaaagaagcggtggaacaggataacggcaacgataaa

SEQ ID NO: 23 - DNA, 522 bp, Drosophila melanogaster
atgcgcagcctgccgatgttttggcgcatggcggaagaaatggcgcgcatgccgcgcctgagcagcccgtttcatgcgttttttcatgaaccgccggtgtggagcgtggcgctgccgcgcaactggcagcatattgcgcgctggcaggaacaggaactggcgccgccggcgaccgtgaacaaagatggctataaactgaccctggatgtgaaagattatagcgaactgaaagtgaaagtgctggatgaaagcgtggtgctggtggaagcgaaaagcgaacagcaggaagcggaacagggcggctatagcagccgccattttctgggccgctatgtgctgccggatggctatgaagcggataaagtgagcagcagcctgagcgatgatggcgtgctgaccattagcgtgccgaacccgccgggcgtgcaggaaaccctgaaagaacgcgaagtgaccattgaacagaccggcgaaccggcgaaaaaaagcgcggaagaaccgaaagataaaaccgcgagccag

SEQ ID NO: 24 - DNA, 522 bp, Anser cygnoides; identical to SEQ ID NO: 20

SEQ ID NO: 25 - DNA, 519 bp, Artificial Sequence
  artificial polynucleotide
atggatattaccattcagcatccgtggtttaaacgcgcgctgggcccgctgattccggaacgcctgtttgatcagttttttggcagcggcctgctgagctatgatctgctgccgctgtttgaagaaaccattgaaccgtattatcgccaggaactgtttcgcgaagtgctgagcgaaggcattgaaagcgtgcgcgaagatcgcgataaatttaccattatgctggatgtgaaacattttgaaccgagcgatctggaagtgaaaattattgatgattttgtgagcattcatggcaaacatgaaagccgccaggatgatcatggctatattgaacgcagctttcatcgccgctatcgcctgccggcgaacgtggatcaggaagcgattacctgcgaactggaaggcgatggcatgctgacctttgaaggcccgaaagtgccggaaaacatggatccgacccatgaaagccgcccgattccggtggaacgcagcagcaaaccgaccgaagcgccggaagaa

SEQ ID NO: 26 - DNA, 519 bp, Artificial Sequence
  artificial polynucleotide
atggatattaccattcagcatccgtggtttaaacgcgcgctgggcccgctgattccggaacgcctgtttgatcagttttttggcagcggcctgctgagctatgatctgctgccgctgtttgaagaaaccattgaaccgtattatcgccaggaactgtttcgcgaagtgctgagcgaaggcattgaaagcgtgcgcgaagatcgcagcaaatttaccattatgctggatgtgaaacattttgaaccgagcgatctggaagtgaaaattattgatgattttgtgagcattcatggcaaacatgaaagccgccaggatgatcatggctatattgaacgcagctttcatcgccgctatcgcctgccggaaaacgtggatcaggaagcgattacctgcgaactggaagaagatggcatgctgacctttgaaggcccgaaagtgcaggcgaacatggatccggaacatgaaagccgcccgattccggtggaacgcagcagcaaaccgaccgaagcgccggaagaa

SEQ ID NO: 27 - DNA, 447 bp, Artificial Sequence
  artificial polynucleotide
cgcgcgctgggcccgctgattccggaacgcctgtttgatcagttttttggcagcggcctgctgagctatgatctgctgccgctgtttgaagaaaccattgaaccgtattatcgccaggaactgtttcgcgaagtgctgagcgaaggcattgaaagcgtgcgcgaagatcgcgataaatttaccattatgctggatgtgaaacattttgaaccgagcgatctggaagtgaaaattattgatgattttgtgagcattcatggcaaacatgaaagccgccaggatgatcatggctatattgaacgcagctttcatcgccgctatcgcctgccggcgaacgtggatcaggaagcgattacctgcgaactggaaggcgatggcatgctgacctttgaaggcccgaaagtgccggaaaacatggatccgacccatgaaagccgcccgattccg

SEQ ID NO: 28 - DNA, 522 bp, Artificial Sequence
  artificial polynucleotide
atgagcattaccattcataacccgctgattcgccgcccgctgtttgattggctggcgccggatcgcatttttagccagatttttggcgaacatctgcaggaagatgaactgctgccggcggatccggatctggatccgtttctgatgcgcgatccgatttttcgcatgccggattggctggaaaccggcctggatgaaatgcgcctggaaaaaagcaaatttgatgtgaacctgagcgtgaaacattttgatccggaagaactgaaagtgaaagtgctgggcagcatggtggaaattcatggcaaacatgaagaacgccagagcgaacatggctttattgcgcgcgaatttaaccgcaaatatcgcattccggcgagcgtgagcccgctgaccattaccgatgatctggatctgagcggcgtgctgaccgtggatgcgccgcgcaaacaggatagcgtgccggaacgcgatattccgattacccgcgaagaaaaaccggcgattgcgggcgcgcagcgcaaa

SEQ ID NO: 29 - DNA, 519 bp, Artificial Sequence
  artificial polynucleotide
atggatgtgaccattcagcatccgtggtttaaacgcaccctgggcccgttttatccggaacgcctgtttgatcagttttttggcagcggcctgtttagctatgatctgctgccgtttctggaagaaaccattgaaccgtattatcgccaggaactgtttcgcaccgtgctggatgaaggcattgaaagcgtgcgcgaagatcgcgataaatttgtgatttttctggatgtgaaacattttgaaccgagcgatctgaccgtgaaagtgcaggatgattttgtgagcattcatggcaaacataacagccgccaggatgatcatggctatattgaacgcagctttcatcgccgctatcgcctgccggaaaacgtggatcaggaagcgctggaatgcgaactggaagcggatggcatgctgaccttttgcggcccgaaaattcagaccggcctggatgcgacccatgcgagccgcgcgattccggtggaacgcagcagcaaaccgaccgaagcgccggaagaa

SEQ ID NO: 30 - DNA, 558 bp, Artificial Sequence
  artificial polynucleotide
atggcgaacattccgctgctgctgagcctggcggtggtgctgggccgcatgagcatggatccgttttatgaaccgtattattgccagcgccagcgcaacccgtatctggcgctggatggcccgatggaacagcagctgcgccagctggaaaaacaggatggcgcgagcagcggcagcagcggcgcggatagcaaaattggcaaagtgggctttcaggattgcatggtggatagccattttaaaccgagcgaactggatgataaagatcaggtgaacagcgatctggatgaaggcaaccatgaagaacgcgaagtggtgcatggctttattacccgccattttgatcgccgctatgcgctgccgccgggctatgaagcggtgaaagatgcgagcaccctgagcagcgtgggcgatctgaccattaaagatccgaaaccgccggcgattgaagtgaaaggcaacgaacgcattgatcagattcagcaggatggcccggcgcatctgaacgataaagaaaacccgaaagaagcggatgaacaggtgaacggcaacgtgaaa

SEQ ID NO: 31 - DNA, 522 bp, Artificial Sequence
  artificial polynucleotide
atgcgcctgagcccgatgttttggcgcatggcggaagaaatggcgcgcatgccgcgcagcctgctgccgtttcatgcgttttttcatgaaccgccggattggctggatgcgagcccgcgcaactggcagcatattgcgcgctggcaggaacaggaaagcgcgccgccggcgaccgataacaaagtgggctataaaagcaccagcgtggataaagtgtatctggaaagcaaagataaagatagcgtggaactggatgatagcgatgaagcgaaactggaacagcaggaagcggaacagggcggctatctgctgcgccattttagcggccgctatgatagcccggtgggctatgaagcggtgaaagatctgctgctgagcctggtggtgggcgatagcaccattctggatccgaacccgccgggcgatcaggaaaccagcaaagaacgcgaagataccattgaacagaccggcgaaccggcgaaaaaactggcggaagaaccgaaagtgaaaaccgcgctgcag

SEQ ID NO: 32 - DNA, 522 bp, Artificial Sequence; identical to SEQ ID NO: 28
  artificial polynucleotide

SEQ ID NO: 33 - DNA, 50 bp, Anser cygnoides
ggggggcatatggacattaccatccagcacccctggttcaagcgcgctct

SEQ ID NO: 34 - DNA, 39 bp, Anser cygnoides
ggggggaagcttttactcctcaggcgcctcggtgggctt

SEQ ID NO: 35 - DNA, 32 bp, Artificial Sequence
  artificial polynucleotide
cctctgttcgaggagactatcgagccctacta

SEQ ID NO: 36 - DNA, 32 bp, Artificial Sequence
  artificial polynucleotide
tagtagggctcgatagtctcctcgaacagagg

SEQ ID NO: 37 - DNA, 64 bp, Artificial Sequence
  artificial polynucleotide
accggcaggagctgttccgcgaggtgctgtcggagggcattgagtcggtgagggaggaccggga

SEQ ID NO: 38 - DNA, 64 bp, Artificial Sequence
  artificial polynucleotide
tcccggtcctccctcaccgactcaatgccctccgacagcacctcgcggaacagctcctgccggt

SEQ ID NO: 39 - DNA, 52 bp, Artificial Sequence
  artificial polynucleotide
actatgctggacgtaaaacactttgagccttcggacctggaggtgaagatta

SEQ ID NO: 40 - DNA, 52 bp, Artificial Sequence
  artificial polynucleotide
taatcttcacctccaggtccgaaggctcaaagtgttttacgtccagcatgat

SEQ ID NO: 41 - DNA, 33 bp, Artificial Sequence
  artificial polynucleotide
aagattatcgacgactttgtgtcgatccatggc

SEQ ID NO: 42 - DNA, 33 bp, Artificial Sequence
  artificial polynucleotide
gccatggatcgacacaaagtcgtcgataatctt

SEQ ID NO: 43 - DNA, 57 bp, Artificial Sequence
  artificial polynucleotide
ggcaagcacgagtcgagacaggacgaccacggctacatcgagcggtcgtttcaccgc

SEQ ID NO: 44 - DNA, 57 bp, Artificial Sequence
  artificial polynucleotide
gcggtgaaacgaccgctcgatgtagccgtggtcgtcctgtctcgactcgtgcttgcc

SEQ ID NO: 45 - DNA, 41 bp, Artificial Sequence
  artificial polynucleotide
gcggaccaggaggccatcacctgcgagctggagggcgacgg

SEQ ID NO: 46 - DNA, 41 bp, Artificial Sequence
  artificial polynucleotide
ccgtcgccctccagctcgcaggtgatggcctcctggtccac

SEQ ID NO: 47 - DNA, 54 bp, Artificial Sequence
  artificial polynucleotide
ttcgaccagtttttcggatcgggtctgctgtcgtatgacctgctgcctctgttc

SEQ ID NO: 48 - DNA, 39 bp, Artificial Sequence
  artificial polynucleotide
ggggaccttggggccctcgaaggtcagcatgccgtcgcc

SEQ ID NO: 49 - DNA, 57 bp, Artificial Sequence
  artificial polynucleotide
ttcaagcgcgctctgggacccctgattccagagcgtctgttcgaccagtttttcgga

SEQ ID NO: 50 - DNA, 55 bp, Artificial Sequence
  artificial polynucleotide
cacggggatgggcctcgactcgtgggtggggtccatgttctcggggaccttgggg

SEQ ID NO: 51 - DNA, 18 bp, Artificial Sequence
  artificial polynucleotide
atggacattaccatccag

SEQ ID NO: 52 - DNA, 60 bp, Artificial Sequence
  artificial polynucleotide
aagcttttactcctcaggcgcctcggtgggcttcgacgaccgctccacggggatgggcct